European Patent Application EP 4 375 670 A1, published May 29, 2024. Title: 조절 T 세포 표면 항원의 에피토프 및 이에 특이적으로 결합하는 항체. Applicant: 주식회사 굳티셀. Application KR. The sequence listing filed with the application follows.

SEQUENCE LISTING (93 sequences)

SEQ ID NO: 1 - protein, 1093 aa, Homo sapiens [sequence omitted]

SEQ ID NO: 2 - DNA, 3282 bp, Homo sapiens
  source 1..3282: mol_type = genomic DNA
atggcgcggccggtccggggagggctcggggccccgcgccgctcgccttgccttctccttctctggctgcttttgcttcggctggagccggtgaccgccgcggccggcccgcgggcgccctgcgcggccgcctgcacttgcgctggggactcgctggactgcggtgggcgcgggctggctgcgttgcccggggacctgccctcctggacgcggagcctaaacctgagttacaacaaactctctgagattgaccctgctggttttgaggacttgccgaacctacaggaagtgtacctcaataataatgagttgacagcggtaccatccctgggcgctgcttcatcacatgtcgtctctctctttctgcagcacaacaagattcgcagcgtggaggggagccagctgaaggcctacctttccttagaagtgttagatctgagtttgaacaacatcacggaagtgcggaacacctgctttccacacggaccgcctataaaggagctcaacctggcaggcaatcggattggcaccctggagttgggagcatttgatggtctgtcacggtcgctgctaactcttcgcctgagcaaaaacaggatcacccagcttcctgtaagagcattcaagctacccaggctgacacaactggacctcaatcggaacaggattcggctgatagagggcctcaccttccaggggctcaacagcttggaggtgctgaagcttcagcgaaacaacatcagcaaactgacagatggggccttctggggactgtccaagatgcatgtgctgcacctggagtacaacagcctggtagaagtgaacagcggctcgctctacggcctcacggccctgcatcagctccacctcagcaacaattccatcgctcgcattcaccgcaagggctggagcttctgccagaagctgcatgagttggtcctgtccttcaacaacctgacacggctggacgaggagagcctggccgagctgagcagcctgagtgtcctgcgtctcagccacaattccatcagccacattgcggagggtgccttcaagggactcaggagcctgcgagtcttggatctggaccataacgagatttcgggcacaatagaggacacgagcggcgccttctcagggctcgacagcctcagcaagctgactctgtttggaaacaagatcaagtctgtggctaagagagcattctcggggctggaaggcctggagcacctgaaccttggagggaatgcgatcagatctgtccagtttgatgcctttgtgaagatgaagaatcttaaagagctccatatcagcagcgacagcttcctgtgtgactgccagctgaagtggctgcccccgtggctaattggcaggatgctgcaggcctttgtgacagccacctgtgcccacccagaatcactgaagggtcagagcattttctctgtgccaccagagagtttcgtgtgcgatgacttcctgaagccacagatcatcacccagccagaaaccaccatggctatggtgggcaaggacatccggtttacatgctcagcagccagcagcagcagctcccccatgacctttgcctggaagaaagacaatgaagtcctgaccaatgcagacatggagaactttgtccacgtccacgcgcaggacggggaagtgatggagtacaccaccatcctgcacctccgtcaggtcactttcgggcacgagggccgctaccaatgtgtcatcaccaaccactttggctccacctattcacataaggccaggctcaccgtgaatgtgttgccatcattcaccaaaacgccccacgacataaccatccggaccaccaccatggcccgcctcgaatgtgctgccacaggtcacccaaaccctcagattgcctggcagaaggatggaggcacggatttccccgctgcccgtgagcgacgcatgcatgtcatgccggatgacgacgtgtttttcatcactgatgtgaaaatagatgacgcaggggtttacagctgtactgctcagaactcagccggttctatttcagctaatgccaccctgactgtcctagagaccccatccttggtggtccccttggaagaccgtgtggtatctgtgggagaaacagtggccctccaatgcaaagccacggggaaccctccgccccgcatcacctggttcaagggggaccgcccgctgagcctcactgagcggcaccacttgacccctgacaaccagctcctggtggttcagaacgtggtggcagaggatgcgggccgatatacctgtgagatgtccaacaccctgggcacggagcgagctcacagccagctgagcgtcctgcccgcagcaggctgcaggaaggatgggaccacggtaggcatcttcaccattgctgtcgtgagcagcatcgtcctgacgtcactggtctgggtgtgcatcatctaccagaccaggaagaagagtgaagagtacagtgtcaccaacacagatgaaaccgtcgtgccaccagatgttccaagctacctctcttctcaggggaccctttctgaccgacaagaaaccgtggtcaggaccgagggtggccctcaggccaatgggcacattgagagcaatggtgtgtgtccaagagatgcaagccactttccagagcccgacactcacagcgttgcctgcaggcagccaaagctctgtgctgggtctgcgtatcacaaagagccgtggaaagcgatggagaaagctgaagggacacctgggccacataagatggaacacggtggccgggtcgtatgcagtgactgcaacaccgaagtggactgttactccaggggacaagccttccacccccagcctgtgtccagagacagcgcacagccaagtgcgccaaatggcccggagccgggtgggagtgaccaagagcattctccacatcaccagtgcagcaggactgccgctgggtcctgccccgagtgccaagggtcgctctaccccagtaaccacgatagaatgctgacggctgtgaagaaaaagccaatggcatctctagatgggaaaggggattcttcctggactttagcaaggttgtatcacccggactccacagagctacagcctgcatcttcattaacttcaggcagtccagagcgcgcggaagcccagtacttgcttgtttccaatggccacctccccaaagcatgtgacgccagtcccgagtccacgccactgacaggacagctccccgggaaacagagggtgccactgctgttggcaccaaaaagctag

SEQ ID NO: 3 - protein, 1091 aa, Mus musculus
MARPGPGVLGAPRLAPRLLLWLLLLLLQWPESAGAQAGPRAPCAAACTCAGDSLDCSGRGLATLPRDLPSWTRSLNLSYNRLSEIDSAAFEDLTNLQEVYLNSNELTAIPSLGTASIGVVSLFLQHNKILSVDGSQLKSYLSLEVLDLSSNNITEIRSSCFPNGLRIRELNLASNRISILESGAFDGLSRSLLTLRLSKNRITQLPVKAFKLPRLTQLDLNRNRIRLIEGLTFQGLDSLEVLRLQRNNISRLTDGAFWGLSKMHVLHLEYNSLVEVNSGSLYGLTALHQLHLSNNSISRIQRDGWSFCQKLHELILSFNNLTRLDEESLAELSSLSILRLSHNAISHIAEGAFKGLKSLRVLDLDHNEISGTIEDTSGAFTGLDNLSKLTLFGNKIKSVAKRAFSGLESLEHLNLGENAIRSVQFDAFAKMKNLKELYISSESFLCDCQLKWLPPWLMGRMLQAFVTATCAHPESLKGQSIFSVLPDSFVCDDFPKPQIITQPETTMAVVGKDIRFTCSAASSSSSPMTFAWKKDNEVLANADMENFAHVRAQDGEVMEYTTILHLRHVTFGHEGRYQCIITNHFGSTYSHKARLTVNVLPSFTKIPHDIAIRTGTTARLECAATGHPNPQIAWQKDGGTDFPAARERRMHVMPDDDVFFITDVKIDDMGVYSCTAQNSAGSVSANATLTVLETPSLAVPLEDRVVTVGETVAFQCKATGSPTPRITWLKGGRPLSLTERHHFTPGNQLLVVQNVMIDDAGRYTCEMSNPLGTERAHSQLSILPTPGCRKDGTTVGIFTIAVVCSIVLTSLVWVCIIYQTRKKSEEYSVTNTDETIVPPDVPSYLSSQGTLSDRQETVVRTEGGHQANGHIESNGVCLRDPSLFPEVDIHSTTCRQPKLCVGYTREPWKVTEKADRTAAPHTTAHSGSAVCSDCSTDTAYHPQPVPRDSGQPGTASSQELRQHDREYSPHHPYSGTADGSHTLSGGSLYPSNHDRILPSLKNKAASADGNGDSSWTLAKLHEADCIDLKPSPTLASGSPELMEDAISTEAQHLLVSNGHLPKACDSSPESVPLKGQITGKRRGPLLLAPRS

SEQ ID NO: 4 - DNA, 3276 bp, Mus musculus
  source 1..3276: mol_type = genomic DNA
atggcgcggcccggtccgggagtgctcggagccccgcgccttgcgcctcgccttctgctctggctgctcttgctgctactgcaatggccggagtcagcgggcgcccaggctcgcccgcgggccccctgcgcggccgcctgcacttgcgccgggaactcgctggactgcagtgggcgcgggctggcgacgctgccccgggacctgccctcctggacgcgcagcctaaacctgagttataacagactctccgagatcgactctgctgcttttgaggacttgacgaatctgcaggaagtgtacctcaacagcaatgagctgacagccataccatcactgggcactgcttccataggagttgtctctctctttttgcagcacaacaagatccttagtgtggatgggagccagctgaagtcgtacctgtccttggaagtgctggatctgagttccaacaacatcacggaaattcggagctcctgtttcccgaacggcctgcgtataagggaactcaacttggcgagcaaccgcatcagcatcctggagtctggagcatttgatggtctgtcgcggtcactgctgactctccgtctgagcaaaaacaggatcacccagcttcctgtgaaagcgttcaagctacccaggctgacacaactagacctgaatcggaatcggattcggctgattgaaggcctcacgttccaggggctcgacagcttagaggtgctgaggcttcagaggaacaacatcagcaggctgacggacggggccttctgggggctgtctaagatgcacgtgctgcacctggagtacaacagtctggtggaagtgaacagtggctccctctatggcctcacagccctgcaccagctgcacctcagcaacaactccatctctcgaattcagcgtgatggctggagcttctgccaaaagctgcatgagttgattctgtccttcaacaacctcacgcggctggatgaggagagtctagcggagttgagcagcctcagtatcctgcgcctcagtcacaacgccatcagtcacattgctgaaggcgccttcaagggactcaagagtctgcgggtcttggacctggaccataacgagatctcgggtacaatcgaggataccagtggtgcctttacggggcttgacaacctcagcaagctgactctgtttggaaacaagatcaaatctgtggctaagagagccttctcgggcctggaaagcctggaacacctgaaccttggagagaatgcaatcaggtctgtccagtttgatgcctttgcaaagatgaagaaccttaaagagctctacatcagcagtgagagcttcctgtgtgactgccagctcaagtggctgcccccatggctaatgggtaggatgctgcaggcctttgtgacagccacctgtgcccatccagagtcgctgaagggccagagcattttctcagtgctgccagacagctttgtgtgtgatgactttccaaagccacagatcatcacccagcctgagacgaccatggctgtggtgggcaaggacatccgtttcacatgctccgcagccagcagcagcagctcaccaatgaccttcgcctggaagaaggacaatgaggtcctggccaatgcagacatggagaactttgcccacgtccgtgcacaggacggcgaagtgatggagtataccactatcctgcacctccgtcacgtcacctttgggcacgagggccgctaccagtgtatcatcacaaaccactttggctccacatactcccacaaagccaggctcactgtgaatgtgttgccatcattcactaaaataccccatgacattgccatccggactggcaccacagcccgcctcgagtgtgctgccacgggccaccctaaccctcagattgcctggcagaaggatggaggcaccgatttcccggcagctcgtgagcgacgcatgcatgttatgccagacgatgatgtgttcttcatcactgatgtgaaaatagacgacatgggggtctacagctgcactgcccagaactcggcaggctcggtttcagccaacgctaccctcacagtcttagaaactccatccttggcagtgcctctggaagaccgtgtggtaactgtgggagaaacagtggccttccagtgcaaagcaaccgggagccccacaccacgcatcacctggcttaagggaggtcgcccattgagcctcacagagcgccaccatttcactccaggcaaccagctgctggttgttcagaatgtgatgatagacgatgcagggcggtatacctgtgagatgtctaatcccctgggcactgagcgagcacatagccagctgagcattttacctacccctggctgccggaaggatgggaccaccgtaggcatcttcaccattgctgtggtgtgcagtattgtcctgacctcgctggtgtgggtgtgcatcatctaccagaccaggaagaagagcgaggagtacagcgtcactaacacagatgaaaccattgtgcctccagatgttccaagctacctctcctctcagggaaccctttctgaccggcaggaaactgtggtcaggactgagggtggtcatcaggccaatgggcacattgaaagcaatggtgtgtgtctgagagacccgagcctcttcccagaggtcgacattcatagcactacatgtaggcagcccaagctgtgtgttggatacactagagagccctggaaggtgacggagaaagccgacaggacagctgccccacatacaacagcacacagtggctctgctgtatgtagtgactgcagtactgacacagcctaccatccccagcctgtgcccagagacagtgggcagccaggcacagcgagcagccaagagctcaggcagcatgaccgggaatattctccacaccatccttacagtgggactgcggatgggtctcataccctctctggggggtccctctatccaagcaaccatgacagaatactgccatccttgaagaacaaggcggcgtctgcagatgggaacggagattcctcttggactttagcaaagttacatgaagcagactgcatagacctaaagccttctcctacgttagcttcaggcagcccagagctcatggaagacgccatatctactgaagcccagcacttgcttgtttccaatggccacctccccaaggcctgtgactccagccctgaatctgtgccactgaaagggcagatcactgggaaacggaggggaccactgctattggcaccgagaagctag

SEQ ID NO: 5 - protein, 762 aa, Homo sapiens
AGPRAPCAAACTCAGDSLDCGGRGLAALPGDLPSWTRSLNLSYNKLSEIDPAGFEDLPNLQEVYLNNNELTAVPSLGAASSHVVSLFLQHNKIRSVEGSQLKAYLSLEVLDLSLNNITEVRNTCFPHGPPIKELNLAGNRIGTLELGAFDGLSRSLLTLRLSKNRITQLPVRAFKLPRLTQLDLNRNRIRLIEGLTFQGLNSLEVLKLQRNNISKLTDGAFWGLSKMHVLHLEYNSLVEVNSGSLYGLTALHQLHLSNNSIARIHRKGWSFCQKLHELVLSFNNLTRLDEESLAELSSLSVLRLSHNSISHIAEGAFKGLRSLRVLDLDHNEISGTIEDTSGAFSGLDSLSKLTLFGNKIKSVAKRAFSGLEGLEHLNLGGNAIRSVQFDAFVKMKNLKELHISSDSFLCDCQLKWLPPWLIGRMLQAFVTATCAHPESLKGQSIFSVPPESFVCDDFLKPQIITQPETTMAMVGKDIRFTCSAASSSSSPMTFAWKKDNEVLTNADMENFVHVHAQDGEVMEYTTILHLRQVTFGHEGRYQCVITNHFGSTYSHKARLTVNVLPSFTKTPHDITIRTTTVARLECAATGHPNPQIAWQKDGGTDFPAARERRMHVMPDDDVFFITDVKIDDAGVYSCTAQNSAGSISANATLTVLETPSLVVPLEDRVVSVGETVALQCKATGNPPPRITWFKGDRPLSLTERHHLTPDNQLLVVQNVVAEDAGRYTCEMSNTLGTERAHSQLSVLPAAGCRKDGTTVGIF

SEQ ID NO: 6 - protein, 760 aa, Mus musculus
AQAGPRAPCAAACTCAGDSLDCSGRGLATLPRDLPSWTRSLNLSYNRLSEIDSAAFEDLTNLQEVYLNSNELTAIPSLGAASIGVVSLFLQHNKILSVDGSQLKSYLSLEVLDLSSNNITEIRSSCFPNGLRIRELNLASNRISILESGAFDGLSRSLLTLRLSKNRITQLPVKAFKLPRLTQLDLNRNRIRLIEGLTFQGLDSLEVLRLQRNNISRLTDGAFWGLSKMHVLHLEYNSLVEVNSGSLYGLTALHQLHLSNNSISRIQRDGWSFCQKLHELILSFNNLTRLDEESLAELSSLSILRLSHNAISHIAEGAFKGLKSLRVLDLDHNEISGTIEDTSGAFTGLDNLSKLTLFGNKIKSVAKRAFSGLESLEHLNLGENAIRSVQFDAFAKMKNLKELYISSESFLCDCQLKWLPPWLMGRMLQAFVTATCAHPESLKGQSIFSVLPDSFVCDDFPKPQIITQPETTMAVVGKDIRFTCSAASSSSSPMTFAWKKDNEVLANADMENFAHVRAQDGEVMEYTTILHLRHVTFGHEGRYQCIITNHFGSTYSHKARLTVNVLPSFTKIPHDIAIRTGTTARLECAATGHPNPQIAWQKDGGTDFPAARERRMHVMPDDDVFFITDVKIDDMGVYSCTAQNSAGSVSANATLTVLETPSLAVPLEDRVVTVGETVAFQCKATGSPTPRITWLKGGRPLSLTERHHFTPGNQLLVVQNVMIDDAGRYTCEMSNPLGTERAHSQLSILPTPGCRKDGTT

SEQ ID NO: 7 - DNA, 24 bp, synthetic construct
  source 1..24: mol_type = other DNA
gacggaattcagtgaggagaacct

SEQ ID NO: 8 - DNA, 24 bp, synthetic construct
  source 1..24: mol_type = other DNA
caactggtagtggcagcttgtagg

SEQ ID NO: 9 - DNA, 24 bp, synthetic construct
  source 1..24: mol_type = other DNA
tcacaaggaacattgtctgaacca

SEQ ID NO: 10 - DNA, 24 bp, synthetic construct
  source 1..24: mol_type = other DNA
gcctgatctaacacatcctcctca

SEQ ID NO: 11 - DNA, 24 bp, synthetic construct
  source 1..24: mol_type = other DNA
cagcaccttgagctgaacagaaac

SEQ ID NO: 12 - DNA, 24 bp, synthetic construct
  source 1..24: mol_type = other DNA
ccagcctttggtaatctcggttag

SEQ ID NO: 13 - DNA, 24 bp, synthetic construct
  source 1..24: mol_type = other DNA
ctttcacctatcccacccttatcc

SEQ ID NO: 14 - DNA, 24 bp, synthetic construct
  source 1..24: mol_type = other DNA
attcatctacggtccacactgctc

SEQ ID NO: 15 - DNA, 20 bp, synthetic construct
  source 1..20: mol_type = other DNA
ggcgtcatggtgggcatggg

SEQ ID NO: 16 - DNA, 20 bp, synthetic construct
  source 1..20: mol_type = other DNA
atggcgtggggaagggcgta

SEQ ID NO: 17 - protein, 451 aa, synthetic construct
EVQLLESGGGLVQPGGSLRLSCAASGFTFSGYDMSWVRQAPGKGLEWVSLIYPDSGNKYYADSVKGRFTISRDNSKNTLYLQMNSLRAEDTAVYYCARDAGLSWAGAFDYWGQGTLVTVSSASTTAPSVYPLAPVCGDTTGSSVTLGCLVKGYFPEPVTLTWNSGSLSSGVHTFPAVLQSDLYTLSSSVTVTSSTWPSQSITCNVAHPASSTKVDKKIEPRGPTIKPCPPCKCPAPNLLGGPSVFIFPPKIKDVLMISLSPIVTCVVVDVSEDDPDVQISWFVNNVEVHTAQTQTHREDYNSTLRVVSALPIQHQDWMSGKEFKCKVNNKDLPAPIERTISKPKGSVRAPQVYVLPPPEEEMTKKQVTLTCMVTDFMPEDIYVEWTNNGKTELNYKNTEPVLDSDGSYFMYSKLRVEKKNWVERNSYSCSVVHEGLHNHHTTKSFSRTPGK

SEQ ID NO: 18 - protein, 217 aa, synthetic construct
QSVLTQPPSASGTPGQRVTISCSGSSSNIGSNYVTWYQQLPGTAPKLLIYSDSHRPSGVPDRFSGSKSGTSASLAISGLQSEDEADYYCGSWDYSLSAYVFGGGTKLTVLRTVAAPTVSIFPPSSEQLTSGGASVVCFLNNFYPKDINVKWKIDGSERQNGVLNSWTDQDSKDSTYSMSSTLTLTKDEYERHNSYTCEATHKTSTSPIVKSFNRNEC

SEQ ID NO: 19 - protein, 451 aa, synthetic construct
EVQLLESGGGLVQPGGSLRLSCAASGFTFSNYYMSWVRQAPGKGLEWVSGISPGDSSTYYADSVKGRFTISRDNSKNTLYLQMNSLRAEDTAVYYCAKGLYSNPNEPFDYWGQGTLVTVSSASTTAPSVYPLAPVCGDTTGSSVTLGCLVKGYFPEPVTLTWNSGSLSSGVHTFPAVLQSDLYTLSSSVTVTSSTWPSQSITCNVAHPASSTKVDKKIEPRGPTIKPCPPCKCPAPNLLGGPSVFIFPPKIKDVLMISLSPIVTCVVVDVSEDDPDVQISWFVNNVEVHTAQTQTHREDYNSTLRVVSALPIQHQDWMSGKEFKCKVNNKDLPAPIERTISKPKGSVRAPQVYVLPPPEEEMTKKQVTLTCMVTDFMPEDIYVEWTNNGKTELNYKNTEPVLDSDGSYFMYSKLRVEKKNWVERNSYSCSVVHEGLHNHHTTKSFSRTPGK

SEQ ID NO: 20 - protein, 217 aa, synthetic construct
QSVLTQPPSASGTPGQRVTISCTGSSSNIGSNYVSWYQQLPGTAPKLLIYDDSQRPSGVPDRFSGSKSGTSASLAISGLRSEDEADYYCGTWDYSLNGYVFGGGTKLTVLRTVAAPTVSIFPPSSEQLTSGGASVVCFLNNFYPKDINVKWKIDGSERQNGVLNSWTDQDSKDSTYSMSSTLTLTKDEYERHNSYTCEATHKTSTSPIVKSFNRNEC

SEQ ID NO: 21 - protein, 457 aa, synthetic construct
EVQLLESGGGLVQPGGSLRLSCAASGFTFSSYDMSWVRQAPGKGLEWVSGISPDGSNIYYADSVKGRFTISRDNSKNTLYLQMNSLRAEDTAVYYCAKVGLRCRYEACSYAYGMDVWGQGTLVTVSSASTTAPSVYPLAPVCGDTTGSSVTLGCLVKGYFPEPVTLTWNSGSLSSGVHTFPAVLQSDLYTLSSSVTVTSSTWPSQSITCNVAHPASSTKVDKKIEPRGPTIKPCPPCKCPAPNLLGGPSVFIFPPKIKDVLMISLSPIVTCVVVDVSEDDPDVQISWFVNNVEVHTAQTQTHREDYNSTLRVVSALPIQHQDWMSGKEFKCKVNNKDLPAPIERTISKPKGSVRAPQVYVLPPPEEEMTKKQVTLTCMVTDFMPEDIYVEWTNNGKTELNYKNTEPVLDSDGSYFMYSKLRVEKKNWVERNSYSCSVVHEGLHNHHTTKSFSRTPGK

SEQ ID NO: 22 - protein, 217 aa, synthetic construct
QSVLTQPPSASGTPGQRVTISCSGSSSNIGSNYVSWYQQLPGTAPKLLIYSDSHRPSGVPDRFSGSKSGTSASLAISGLRSEDEADYYCATWDSSLNGYVFGGGTKLTVLRTVAAPTVSIFPPSSEQLTSGGASVVCFLNNFYPKDINVKWKIDGSERQNGVLNSWTDQDSKDSTYSMSSTLTLTKDEYERHNSYTCEATHKTSTSPIVKSFNRNEC

SEQ ID NO: 23 - protein, 451 aa, synthetic construct
EVQLLESGGGLVQPGGSLRLSCAASGFTFSNYDMSWVRQAPGKGLEWVSSISPSSGSIYYADSVKGRFTISRDNSKNTLYLQMNSLRAEDTAVYYCAKDLDAFWRPSFDYWGQGTLVTVSSASTTAPSVYPLAPVCGDTTGSSVTLGCLVKGYFPEPVTLTWNSGSLSSGVHTFPAVLQSDLYTLSSSVTVTSSTWPSQSITCNVAHPASSTKVDKKIEPRGPTIKPCPPCKCPAPNLLGGPSVFIFPPKIKDVLMISLSPIVTCVVVDVSEDDPDVQISWFVNNVEVHTAQTQTHREDYNSTLRVVSALPIQHQDWMSGKEFKCKVNNKDLPAPIERTISKPKGSVRAPQVYVLPPPEEEMTKKQVTLTCMVTDFMPEDIYVEWTNNGKTELNYKNTEPVLDSDGSYFMYSKLRVEKKNWVERNSYSCSVVHEGLHNHHTTKSFSRTPGK

SEQ ID NO: 24 - protein, 217 aa, synthetic construct
QSVLTQPPSASGTPGQRVTISCTGSSSNIGNNNVNWYQQLPGTAPKLLIYSDSHRPSGVPDRFSGSKSGTSASLAISGLRSEDEADYYCGSWDDSLSAYVFGGGTKLTVLRTVAAPTVSIFPPSSEQLTSGGASVVCFLNNFYPKDINVKWKIDGSERQNGVLNSWTDQDSKDSTYSMSSTLTLTKDEYERHNSYTCEATHKTSTSPIVKSFNRNEC

SEQ ID NO: 25 - protein, 457 aa, synthetic construct
EVQLLESGGGLVQPGGSLRLSCAASGFTFSDYDMSWVRQVPGKGLEWVSWISHGGGSIYYADSVKGRFTISRDNSKNTLYLQMNSLRAEDTAVYYCARGLGLCKTGLCYYYDAMDVWGQGTLVTVSSASTTAPSVYPLAPVCGDTTGSSVTLGCLVKGYFPEPVTLTWNSGSLSSGVHTFPAVLQSDLYTLSSSVTVTSSTWPSQSITCNVAHPASSTKVDKKIEPRGPTIKPCPPCKCPAPNLLGGPSVFIFPPKIKDVLMISLSPIVTCVVVDVSEDDPDVQISWFVNNVEVHTAQTQTHREDYNSTLRVVSALPIQHQDWMSGKEFKCKVNNKDLPAPIERTISKPKGSVRAPQVYVLPPPEEEMTKKQVTLTCMVTDFMPEDIYVEWTNNGKTELNYKNTEPVLDSDGSYFMYSKLRVEKKNWVERNSYSCSVVHEGLHNHHTTKSFSRTPGK

SEQ ID NO: 26 - protein, 217 aa, synthetic construct
QSVLTQPPSASGTPGQRVTISCTGSSSNIGNNSVTWYQQLPGTAPKLLIYADNNRPSGVPDRFSGSKSGTSASLAISGLRSEDEADYYCAAWDSSLSAYVFGGGTKLTVLRTVAAPTVSIFPPSSEQLTSGGASVVCFLNNFYPKDINVKWKIDGSERQNGVLNSWTDQDSKDSTYSMSSTLTLTKDEYERHNSYTCEATHKTSTSPIVKSFNRNEC

SEQ ID NO: 27 - protein, 446 aa, synthetic construct
EVQLLESGGGLVQPGGSLRLSCAASGFTFSDYYMSWVRQAPGKGLEWVSGISHDSGSKYYADSVKGRFTISRDNSKNTLYLQMNSLRAEDTAVYYCARHWTTFDYWGQGTLVTVSSASTTAPSVYPLAPVCGDTTGSSVTLGCLVKGYFPEPVTLTWNSGSLSSGVHTFPAVLQSDLYTLSSSVTVTSSTWPSQSITCNVAHPASSTKVDKKIEPRGPTIKPCPPCKCPAPNLLGGPSVFIFPPKIKDVLMISLSPIVTCVVVDVSEDDPDVQISWFVNNVEVHTAQTQTHREDYNSTLRVVSALPIQHQDWMSGKEFKCKVNNKDLPAPIERTISKPKGSVRAPQVYVLPPPEEEMTKKQVTLTCMVTDFMPEDIYVEWTNNGKTELNYKNTEPVLDSDGSYFMYSKLRVEKKNWVERNSYSCSVVHEGLHNHHTTKSFSRTPGK

SEQ ID NO: 28 - protein, 217 aa, synthetic construct
QSVLTQPPSASGTPGQRVTISCSGSSSNIGSNNVTWYQQLPGTAPKLLIYANSNRPSGVPDRFSGSKSGTSASLAISGLRSEDEADYYCGAWDYSLSAYVFGGGTKLTVLRTVAAPTVSIFPPSSEQLTSGGASVVCFLNNFYPKDINVKWKIDGSERQNGVLNSWTDQDSKDSTYSMSSTLTLTKDEYERHNSYTCEATHKTSTSPIVKSFNRNEC

SEQ ID NO: 29 - protein, 457 aa, synthetic construct
EVQLLESGGGLVQPGGSLRLSCAASGFTFSNYAMSWVRQAPGKGLEWVSAIYPGGGSIYYADSVKGRFTISRDNSKNTLYLQMNSLRAEDTAVYYCARDILPCPWGRCYYDYAMDVWGQGTLVTVSSASTTAPSVYPLAPVCGDTTGSSVTLGCLVKGYFPEPVTLTWNSGSLSSGVHTFPAVLQSDLYTLSSSVTVTSSTWPSQSITCNVAHPASSTKVDKKIEPRGPTIKPCPPCKCPAPNLLGGPSVFIFPPKIKDVLMISLSPIVTCVVVDVSEDDPDVQISWFVNNVEVHTAQTQTHREDYNSTLRVVSALPIQHQDWMSGKEFKCKVNNKDLPAPIERTISKPKGSVRAPQVYVLPPPEEEMTKKQVTLTCMVTDFMPEDIYVEWTNNGKTELNYKNTEPVLDSDGSYFMYSKLRVEKKNWVERNSYSCSVVHEGLHNHHTTKSFSRTPGK

SEQ ID NO: 30 - protein, 217 aa, synthetic construct
QSVLTQPPSASGTPGQRVTISCSDSSSNIGSNTVSWYQQLPGTAPKLLIYADNNRPSGVPDRFSGSKSGTSASLAISGLRSEDEADYYCGTWDYSLSGYVFGGGTKLTVLRTVAAPTVSIFPPSSEQLTSGGASVVCFLNNFYPKDINVKWKIDGSERQNGVLNSWTDQDSKDSTYSMSSTLTLTKDEYERHNSYTCEATHKTSTSPIVKSFNRNEC

SEQ ID NO: 31 - protein, 457 aa, synthetic construct
EVQLLESGGGLVQPGGSLRLSCAASGFTFSNYAMSWVRQAPGKGLEWVSVISHGGGSTYYADSVKGRFTISRDNSKNTLYLQMNSLRAEDTAVYYCARVISNCHLGVCYYSNGMDVWGQGTLVTVSSASTTAPSVYPLAPVCGDTTGSSVTLGCLVKGYFPEPVTLTWNSGSLSSGVHTFPAVLQSDLYTLSSSVTVTSSTWPSQSITCNVAHPASSTKVDKKIEPRGPTIKPCPPCKCPAPNLLGGPSVFIFPPKIKDVLMISLSPIVTCVVVDVSEDDPDVQISWFVNNVEVHTAQTQTHREDYNSTLRVVSALPIQHQDWMSGKEFKCKVNNKDLPAPIERTISKPKGSVRAPQVYVLPPPEEEMTKKQVTLTCMVTDFMPEDIYVEWTNNGKTELNYKNTEPVLDSDGSYFMYSKLRVEKKNWVERNSYSCSVVHEGLHNHHTTKSFSRTPGK

SEQ ID NO: 32 - protein, 217 aa, synthetic construct
QSVLTQPPSASGTPGQRVTISCSGSSSNIGNNDVYWYQQLPGTAPKLLIYSDSQRPSGVPDRFSGSKSGTSASLAISGLRSEDEADYYCGTWDYSLSGYVFGGGTKLTVLRTVAAPTVSIFPPSSEQLTSGGASVVCFLNNFYPKDINVKWKIDGSERQNGVLNSWTDQDSKDSTYSMSSTLTLTKDEYERHNSYTCEATHKTSTSPIVKSFNRNEC

SEQ ID NO: 33 - protein, 458 aa, synthetic construct
EVQLLESGGGLVQPGGSLRLSCAASGFTFSNYAMSWVRQAPGKGLEWVSVISHGGGSTYYADSVKGRFTISRDNSKNTLYLQMNSLRAEDTAVYYCARVISNCHLGVCYYSNGMDVWGQGTLVTVSSASTKGPSVFPLAPSSKSTSGGTAALGCLVKDYFPEPVTVSWNSGALTSGVHTFPAVLQSSGLYSLSSVVTVPSSSLGTQTYICNVNHKPSNTKVDKKVEPKSCDKTHTCPPCPAPELLGGPSVFLFPPKPKDTLMISRTPEVTCVVVDVSHEDPEVKFNWYVDGVEVHNAKTKPREEQYNSTYRVVSVLTVLHQDWLNGKEYKCKVSNKALPAPIEKTISKAKGQPREPQVYTLPPSREEMTKNQVSLTCLVKGFYPSDIAVEWESNGQPENNYKTTPPVLDSDGSFFLYSKLTVDKSRWQQGNVFSCSVMHEALHNHYTQKSLSLSPGKY

SEQ ID NO: 34 - protein, 217 aa, synthetic construct
QSVLTQPPSASGTPGQRVTISCSGSSSNIGNNDVYWYQQLPGTAPKLLIYSDSQRPSGVPDRFSGSKSGTSASLAISGLRSEDEADYYCGTWDYSLSGYVFGGGTKLTVLRTVAAPSVFIFPPSDEQLKSGTASVVCLLNNFYPREAKVQWKVDNALQSGNSQESVTEQDSKDSTYSLSSTLTLSKADYEKHKVYACEVTHQGLSSPVTKSFNRGEC

SEQ ID NO: 35 - protein, 40 aa, synthetic construct
EVYLNNNELTAVPSLGAASSHVVSLFLQHNKIRSVEGSQL

SEQ ID NO: 36 - protein, 37 aa, synthetic construct
LNNNELTAVPSLGAASSHVVSLFLQHNKIRSVEGSQL

SEQ ID NO: 37 - protein, 14 aa, synthetic construct
LQHNKIRSVEGSQL

SEQ ID NO: 38 - protein, 7 aa, synthetic construct
SVEGSQL

SEQ ID NO: 39 - protein, 5 aa, synthetic construct
LQHNK

SEQ ID NO: 40 - protein, 12 aa, synthetic construct
HNKIRSVEGSQL

SEQ ID NO: 41 - protein, 24 aa, synthetic construct
DLSLNNITEVRNTCFPHGPPIKEL

SEQ ID NO: 42 - protein, 35 aa, synthetic construct
GQSIFSVPPESFVCDDFLKPQIITQPETTMAMVGK

SEQ ID NO: 43 - protein, 9 aa, synthetic construct
AMVGKDIRF

SEQ ID NO: 44 - protein, 5 aa, synthetic construct
AMVGK

SEQ ID NO: 45 - protein, 12 aa, synthetic construct
QCVITNHFGSTY

SEQ ID NO: 46 - protein, 5 aa, synthetic construct
GYDMS

SEQ ID NO: 47 - protein, 17 aa, synthetic construct
LIYPDSGNKYYADSVKG

SEQ ID NO: 48 - protein, 12 aa, synthetic construct
DAGLSWAGAFDY

SEQ ID NO: 49 - protein, 13 aa, synthetic construct
SGSSSNIGSNYVT

SEQ ID NO: 50 - protein, 7 aa, synthetic construct
SDSHRPS

SEQ ID NO: 51 - protein, 11 aa, synthetic construct
GSWDYSLSAYV

SEQ ID NO: 52 - protein, 5 aa, synthetic construct
NYYMS

SEQ ID NO: 53 - protein, 17 aa, synthetic construct
GISPGDSSTYYADSVKG

SEQ ID NO: 54 - protein, 12 aa, synthetic construct
GLYSNPNEPFDY

SEQ ID NO: 55 - protein, 13 aa, synthetic construct
TGSSSNIGSNYVS

SEQ ID NO: 56 - protein, 7 aa, synthetic construct
DDSQRPS

SEQ ID NO: 57 - protein, 11 aa, synthetic construct
GTWDYSLNGYV

SEQ ID NO: 58 - protein, 5 aa, synthetic construct
SYDMS

SEQ ID NO: 59 - protein, 17 aa, synthetic construct
GISPDGSNIYYADSVKG

SEQ ID NO: 60 - protein, 18 aa, synthetic construct
VGLRCRYEACSYAYGMDV

SEQ ID NO: 61 - protein, 13 aa, synthetic construct
SGSSSNIGSNYVS

SEQ ID NO: 62 - protein, 7 aa, synthetic construct
SDSHRPS

SEQ ID NO: 63 - protein, 11 aa, synthetic construct
ATWDSSLNGYV

SEQ ID NO: 64 - protein, 5 aa, synthetic construct
NYDMS

SEQ ID NO: 65 - protein, 17 aa, synthetic construct
SISPSSGSIYYADSVKG

SEQ ID NO: 66 - protein, 12 aa, synthetic construct
DLDAFWRPSFDY

SEQ ID NO: 67 - protein, 13 aa, synthetic construct
TGSSSNIGNNNVN

SEQ ID NO: 68 - protein, 7 aa, synthetic construct
SDSHRPS

SEQ ID NO: 69 - protein, 11 aa, synthetic construct
GSWDDSLSAYV

SEQ ID NO: 70 - protein, 5 aa, synthetic construct
DYDMS

SEQ ID NO: 71 - protein, 17 aa, synthetic construct
WISHGGGSIYYADSVKG

SEQ ID NO: 72 - protein, 18 aa, synthetic construct
GLGLCKTGLCYYYDAMDV

SEQ ID NO: 73 - protein, 13 aa, synthetic construct
TGSSSNIGNNSVT

SEQ ID NO: 74 - protein, 7 aa, synthetic construct
ADNNRPS

SEQ ID NO: 75 - protein, 11 aa, synthetic construct
AAWDSSLSAYV

SEQ ID NO: 76 - protein, 5 aa, synthetic construct
DYYMS

SEQ ID NO: 77 - protein, 17 aa, synthetic construct
GISHDSGSKYYADSVKG

SEQ ID NO: 78 - protein, 7 aa, synthetic construct
HWTTFDY

SEQ ID NO: 79 - protein, 13 aa, synthetic construct
SGSSSNIGSNNVT

SEQ ID NO: 80 - protein, 7 aa, synthetic construct
ANSNRPS

SEQ ID NO: 81 - protein, 11 aa, synthetic construct
GAWDYSLSAYV

SEQ ID NO: 82 - protein, 5 aa, synthetic construct
NYAMS

SEQ ID NO: 83 - protein, 17 aa, synthetic construct
AIYPGGGSIYYADSVKG

SEQ ID NO: 84 - protein, 18 aa, synthetic construct
DILPCPWGRCYYDYAMDV

SEQ ID NO: 85 - protein, 13 aa, synthetic construct
SDSSSNIGSNTVS

SEQ ID NO: 86 - protein, 7 aa, synthetic construct
ADNNRPS

SEQ ID NO: 87 - protein, 11 aa, synthetic construct
GTWDYSLSGYV

SEQ ID NO: 88 - protein, 5 aa, synthetic construct
NYAMS

SEQ ID NO: 89 - protein, 17 aa, synthetic construct
VISHGGGSTYYADSVKG

SEQ ID NO: 90 - protein, 18 aa, synthetic construct
VISNCHLGVCYYSNGMDV

SEQ ID NO: 91 - protein, 13 aa, synthetic construct
SGSSSNIGNNDVY

SEQ ID NO: 92 - protein, 7 aa, synthetic construct
SDSQRPS

SEQ ID NO: 93 - protein, 11 aa, synthetic construct
GTWDYSLSGYV